European Patent Application EP 4 159 758 A1, published April 5, 2023. Title: rhFGF21 fusion protein, polynucleotide encoding rhFGF21 fusion protein, composition containing rhFGF21 fusion protein, and use of rhFGF21 fusion protein. Applicant: JIANGSU KANIONREAL BIOMEDICAL TECHNOLOGY CO., LTD. The sequence listing filed with the application follows.

SEQUENCE LISTING (13 sequences)

SEQ ID NO: 1 - protein, 181 aa, Artificial Sequence
  rhFGF21
HPIPDSSPLLQFGGQVRQRYLYTDDAQQTEAHLEIREDGTVGGAADQSPESLLQLKALKPGVIQILGVKTSRFLCQRPDGALYGSLHFDPEACSFRELLLEDGYNVYQSEAHGLPLHLPGNKSPHRDPAPRGPARFLPLPGLPPALPEPPGILAPQPPDVGSSDPLSMVGPSQGRSPSYAS

SEQ ID NO: 2 - protein, 385 aa, Artificial Sequence
  rhFGF21-(VPGXG)40 fusion protein
HPIPDSSPLLQFGGQVRQRYLYTDDAQQTEAHLEIREDGTVGGAADQSPESLLQLKALKPGVIQILGVKTSRFLCQRPDGALYGSLHFDPEACSFRELLLEDGYNVYQSEAHGLPLHLPGNKSPHRDPAPRGPARFLPLPGLPPALPEPPGILAPQPPDVGSSDPLSMVGPSQGRSPSYASRSVPGAGVPGAGVPGAGVPGAGVPGAGVPGAGVPGAGVPGAGVPGVGVPGVGVPGVGVPGVGVPGVGVPGVGVPGVGVPGVGVPGVGVPGVGVPGVGVPGVGGSVPGAGVPGAGVPGAGVPGAGVPGAGVPGAGVPGAGVPGAGVPGVGVPGVGVPGVGVPGVGVPGVGVPGVGVPGVGVPGVGVPGVGVPGVGVPGVGVPGVG

SEQ ID NO: 3 - DNA, 543 bp, Artificial Sequence
  nucleotide sequence for encoding rhFGF21
catcctattcctgacagctcacccctgttacagtttggcggtcaggttcgtcaacgctatttatacaccgacgacgcacagcaaaccgaagcacacctggaaattcgtgaagacggcaccgttggtggtgcagcagatcaatccccggaatctctgctgcagttaaaagcattaaaaccgggcgttatacagattttaggtgtcaaaacctcccgttttctgtgtcagcggccggacggtgcgctttatggtagcttacactttgatccggaagcctgtagttttcgtgagctgctgctggaggacggttacaatgtttatcaatcagaagcacatggtctgccgttacatctgccgggtaataagagcccgcatcgcgatccggcaccgcgtggtccagccagatttctgcctctgccgggactgccgccggcacttcctgaaccgcctggtattctggcaccgcagccgcctgatgttggttcatctgatcctctgtcaatggttggaccgagccagggacgttctccctcatacgcttct

SEQ ID NO: 4 - DNA, 6 bp, Artificial Sequence
  nucleotide sequence for encoding linker
agatct

SEQ ID NO: 5 - DNA, 6 bp, Artificial Sequence
  nucleotide sequence for encoding linker
ggatcc

SEQ ID NO: 6 - DNA, 1158 bp, Artificial Sequence
  nucleotide sequence for encoding rhFGF21-(VPGXG)40 fusion protein
catcctattcctgacagctcacccctgttacagtttggcggtcaggttcgtcaacgctatttatacaccgacgacgcacagcaaaccgaagcacacctggaaattcgtgaagacggcaccgttggtggtgcagcagatcaatccccggaatctctgctgcagttaaaagcattaaaaccgggcgttatacagattttaggtgtcaaaacctcccgttttctgtgtcagcggccggacggtgcgctttatggtagcttacactttgatccggaagcctgtagttttcgtgagctgctgctggaggacggttacaatgtttatcaatcagaagcacatggtctgccgttacatctgccgggtaataagagcccgcatcgcgatccggcaccgcgtggtccagccagatttctgcctctgccgggactgccgccggcacttcctgaaccgcctggtattctggcaccgcagccgcctgatgttggttcatctgatcctctgtcaatggttggaccgagccagggacgttctccctcatacgcttctagatctgttccgggtgcaggtgttccgggtgccggtgttccgggggcaggtgttcctggtgcgggtgttccgggcgcgggtgttcctggagcgggtgttccaggtgcgggtgtgccgggtgcgggtgtacctggtgttggtgttccgggagttggtgttcctggggttggtgttccaggggttggtgtgccgggggttggtgtcccgggtgttggtgtgcctggtgttggggttccgggtgttggggtgccgggtgttggcgttccgggtgtgggtgttccgggtgtcggtgttccgggtgtaggtggatctgttccgggtgcaggtgttccgggtgccggtgttccgggggcaggtgttcctggtgcgggtgttccgggcgcgggtgttcctggagcgggtgttccaggtgcgggtgtgccgggtgcgggtgtacctggtgttggtgttccgggagttggtgttcctggggttggtgttccaggggttggtgtgccgggggttggtgtcccgggtgttggtgtgcctggtgttggggttccgggtgttggggtgccgggtgttggcgttccgggtgtgggtgttccgggtgtcggtgttccgggtgtaggttga

SEQ ID NO: 7 - DNA, 303 bp, Artificial Sequence
  nucleotide sequence for encoding (VPGXG)20
gttccgggtgcaggtgttccgggtgccggtgttccgggggcaggtgttcctggtgcgggtgttccgggcgcgggtgttcctggagcgggtgttccaggtgcgggtgtgccgggtgcgggtgtacctggtgttggtgttccgggagttggtgttcctggggttggtgttccaggggttggtgtgccgggggttggtgtcccgggtgttggtgtgcctggtgttggggttccgggtgttggggtgccgggtgttggcgttccgggtgtgggtgttccgggtgtcggtgttccgggtgtaggttga

SEQ ID NO: 8 - DNA, 559 bp, Artificial Sequence
  gene for encoding rhFGF21 with restriction site
ggtctcaggtcatcctattcctgacagctcacccctgttacagtttggcggtcaggttcgtcaacgctatttatacaccgacgacgcacagcaaaccgaagcacacctggaaattcgtgaagacggcaccgttggtggtgcagcagatcaatccccggaatctctgctgcagttaaaagcattaaaaccgggcgttatacagattttaggtgtcaaaacctcccgttttctgtgtcagcggccggacggtgcgctttatggtagcttacactttgatccggaagcctgtagttttcgtgagctgctgctggaggacggttacaatgtttatcaatcagaagcacatggtctgccgttacatctgccgggtaataagagcccgcatcgcgatccggcaccgcgtggtccagccagatttctgcctctgccgggactgccgccggcacttcctgaaccgcctggtattctggcaccgcagccgcctgatgttggttcatctgatcctctgtcaatggttggaccgagccagggacgttctccctcatacgcttctagatct

SEQ ID NO: 9 - DNA, 312 bp, Artificial Sequence
  gene for encoding linker-(VPGXG)20
agatctgttccgggtgcaggtgttccgggtgccggtgttccgggggcaggtgttcctggtgcgggtgttccgggcgcgggtgttcctggagcgggtgttccaggtgcgggtgtgccgggtgcgggtgtacctggtgttggtgttccgggagttggtgttcctggggttggtgttccaggggttggtgtgccgggggttggtgtcccgggtgttggtgtgcctggtgttggggttccgggtgttggggtgccgggtgttggcgttccgggtgtgggtgttccgggtgtcggtgttccgggtgtaggtggatcc

SEQ ID NO: 10 - DNA, 10 bp, Artificial Sequence
  restriction site of BsaI
ggtctcaggt

SEQ ID NO: 11 - DNA, 29 bp, Artificial Sequence
  primer P1
ggtctcaggtcatcctattcctgacagct

SEQ ID NO: 12 - DNA, 22 bp, Artificial Sequence
  primer P2
ggatccacctacacccggaaca

SEQ ID NO: 13 - DNA, 25 bp, Artificial Sequence
  primer P3
ggatcctcaacctacacccggaaca